European Patent Application EP 4 116 439 A1, published January 11, 2023. Title: Method for monitoring the gut microbiome status in broiler production. Applicant: Evonik Operations GmbH. The sequence listing filed with the application follows.

SEQUENCE LISTING (4 sequences)

SEQ ID NO: 1 - DNA, 969 bp, C.perfringens
  misc_feature (10)..(10): n is a, c, g, or t
  misc_feature (391)..(396): n is a, c, g, or t
  misc_feature (418)..(420): n is a, c, g, or t
  misc_feature (443)..(443): n is a, c, g, or t
  misc_feature (497)..(497): n is a, c, g, or t
  misc_feature (502)..(502): n is a, c, g, or t
ttgaaaagantaaaaattatttcaattacactagttcttacaagtgtaattagtacaagccttttttcaactcaaactcaagtttttgcaagtgaattaaatgacataaacaaaattgagttgaaaaatctaagtggagaaataataaaagaaaatggaaaggaagctattaaatatacttctagtgataccgcttcacataaaggttggaaggcaactttaagtggaacatttattgaagatcctcattctgataagaaaactgctttattaaatttagaaggatttataccttctgataaacagatttttggttctaaatattacggaaaaatgaaatggcctgaaacttatagaattaatgtaaaaagtgctgatgtaaataataatnnnnnnatagcaaattctattcctaaannnactatagataaaaaagatgtatntaattcaattggttattctataggcggtaatatatctgttgaaggaaaaactgntggtnctggaataaatgcttcatataatgtccaaaatactataagctatgaacaacctgattttagaacaattcaaagaaaagatgatgcaaatttagcatcatgggatataaaatttgttgagactaaggacggttataatatagattcttatcatgctatttatggaaatcaattattcatgaaatcaagattgtataataatggtgataaaaatttcacagatgatagagatttatcaacattaatttctggtggattttcacccaatatggctttagcattaacagcacctaaaaatgctaaagaatctgtaataatagttgaatatcaaagatttgataatgactatattttaaattgggaaactactcaatggcgaggaacaaacaaactttcgtcaacaagtgaatataacgaatttatgtttaaaataaattggcaagatcataaaatagaatattatctgtaa

SEQ ID NO: 2 - DNA, 20 bp, artificial
  Primer (fw)
tacatatcaactagtggtga

SEQ ID NO: 3 - DNA, 20 bp, artificial
  Primer (rev)
attcttgagtttttccatcc

SEQ ID NO: 4 - DNA, 27 bp, artificial
  Probe
tggaacagatgactacatgtattttgg